European Patent Specification EP 2 250 278 B1, published April 5, 2023. Title: METHODS AND COMPOSITIONS RELATED TO PEPTIDES AND PROTEINS WITH C-TERMINAL ELEMENTS. Applicant: Burnham Institute for Medical Research. Application EP09711840.0. The sequence listing filed with the application follows.

SEQUENCE LISTING (164 sequences)

SEQ ID NO: 1 - protein, 7 aa, Artificial Sequence
  REAGENT
  UNSURE 1..7
GGGGGGR

SEQ ID NO: 2 - protein, 7 aa, Artificial Sequence
  REAGENT
  UNSURE 1..7
RPARPAR

SEQ ID NO: 3 - protein, 8 aa, Artificial Sequence
  REAGENT
  UNSURE 1..8
RPARPARA

SEQ ID NO: 4 - protein, 9 aa, Artificial Sequence
  REAGENT
  UNSURE 1..9
CRGDKGPDC

SEQ ID NO: 5 - protein, 14 aa, Artificial Sequence
  REAGENT
  UNSURE 1..14
KLAKLAKKLAKLAK

SEQ ID NO: 6 - protein, 12 aa, Artificial Sequence
  REAGENT
  UNSURE 1..12
CSWRGLENHRMC

SEQ ID NO: 7 - protein, 5 aa, Artificial Sequence
  REAGENT
  UNSURE 1..5
CREKA

SEQ ID NO: 8 - protein, 12 aa, Artificial Sequence
  REAGENT
  UNSURE 1..11
GGGRKKRSTGGG

SEQ ID NO: 9 - protein, 7 aa, Artificial Sequence
  REAGENT
  UNSURE 1..7
GGGRKKR

SEQ ID NO: 10 - protein, 12 aa, Artificial Sequence
  REAGENT
  UNSURE 1..11
GGGLVPRGSGGG

SEQ ID NO: 11 - protein, 7 aa, Artificial Sequence
  REAGENT
  UNSURE 1..7
GGGLVPR

SEQ ID NO: 12 - protein, 13 aa, Artificial Sequence
  REAGENT
  UNSURE 1..12
GGGPCPGRVVGGG

SEQ ID NO: 13 - protein, 8 aa, Artificial Sequence
  REAGENT
  UNSURE 1..8
GGGPCPGR

SEQ ID NO: 14 - protein, 13 aa, Artificial Sequence
  REAGENT
  UNSURE 1..13
GGGPGSGRSAGGG

SEQ ID NO: 15 - protein, 8 aa, Artificial Sequence
  REAGENT
  UNSURE 1..8
GGGPGSGR

SEQ ID NO: 16 - protein, 13 aa, Artificial Sequence
  REAGENT
  UNSURE 1..13
GGGPGSGKSAGGG

SEQ ID NO: 17 - protein, 8 aa, Artificial Sequence
  REAGENT
  UNSURE 1..8
GGGPGSGK

SEQ ID NO: 18 - protein, 10 aa, Artificial Sequence
  REAGENT
  UNSURE 1..10
CGLIIQKNEC

SEQ ID NO: 19 - protein, 7 aa, Artificial Sequence
  REAGENT
  UNSURE 1..7
RXXRXXX

SEQ ID NO: 20 - protein, 11 aa, Artificial Sequence
  REAGENT
  UNSURE 1..11
RXXRAPPRXXX

SEQ ID NO: 21 - protein, 6 aa, Artificial Sequence
  REAGENT
  UNSURE 1..6
CRGDKG

SEQ ID NO: 22 - protein, 5 aa, Artificial Sequence
  REAGENT
  UNSURE 1..5
CRGDK

SEQ ID NO: 23 - protein, 6 aa, Artificial Sequence
  REAGENT
  UNSURE 1..6
RKXXRK

SEQ ID NO: 24 - protein, 6 aa, Artificial Sequence
  REAGENT
  UNSURE 1..6
RKXXRK

SEQ ID NO: 25 - protein, 4 aa, Artificial Sequence
  REAGENT
  UNSURE 1..4
RXXR

SEQ ID NO: 26 - protein, 5 aa, Artificial Sequence
  REAGENT
  UNSURE 1..5
RKXXR

SEQ ID NO: 27 - protein, 7 aa, Artificial Sequence
  REAGENT
  UNSURE 1..7
RGERPPR

SEQ ID NO: 28 - protein, 7 aa, Artificial Sequence
  REAGENT
  UNSURE 1..7
RVTRPPR

SEQ ID NO: 29 - protein, 6 aa, Artificial Sequence
  REAGENT
  UNSURE 1..6
RKXXRK

SEQ ID NO: 30 - protein, 8 aa, Artificial Sequence
  REAGENT
  UNSURE 1..8
CRCDKPRR

SEQ ID NO: 31 - protein, 7 aa, Artificial Sequence
  REAGENT
  UNSURE 1..7
ATWLPPR

SEQ ID NO: 32 - protein, 4 aa, Artificial Sequence
  REAGENT
  UNSURE 1..4
TKPR

SEQ ID NO: 33 - protein, 5 aa, Artificial Sequence
  REAGENT
  UNSURE 1..5
TKPPR

SEQ ID NO: 34 - protein, 14 aa, Artificial Sequence
  REAGENT
  UNSURE 1..14
RPARSGRSAGGSVA

SEQ ID NO: 35 - protein, 14 aa, Artificial Sequence
  REAGENT
  UNSURE 1..14
LNITHRTRRSTSDN

SEQ ID NO: 36 - protein, 15 aa, Artificial Sequence
  REAGENT
  UNSURE 1..15
SVASSRRHKRFAGVV

SEQ ID NO: 37 - protein, 14 aa, Artificial Sequence
  REAGENT
  UNSURE 1..14
KQEGSRTRRSVLIP

SEQ ID NO: 38 - protein, 14 aa, Artificial Sequence
  REAGENT
  UNSURE 1..13
PATNNRARRELPRF

SEQ ID NO: 39 - protein, 15 aa, Artificial Sequence
  REAGENT
  UNSURE 1..15
PQRERRRKKRGLFGA

SEQ ID NO: 40 - protein, 14 aa, Artificial Sequence
  REAGENT
  UNSURE 1..14
RRVVQREKRAVGIG

SEQ ID NO: 41 - protein, 14 aa, Artificial Sequence
  REAGENT
  UNSURE 1..14
LITGGRRTRREAIV

SEQ ID NO: 42 - protein, 15 aa, Artificial Sequence
  REAGENT
  UNSURE 1..15
PSSGSRRHKRFAGIA

SEQ ID NO: 43 - protein, 14 aa, Artificial Sequence
  REAGENT
  UNSURE 1..14
CDSAGRSRRSRRAI

SEQ ID NO: 44 - protein, 13 aa, Artificial Sequence
  REAGENT
  UNSURE 1..13
AAVLRRRRRDAGN

SEQ ID NO: 45 - protein, 14 aa, Artificial Sequence
  REAGENT
  UNSURE 1..14
QIENPRQSRFVLGA

SEQ ID NO: 46 - protein, 14 aa, Artificial Sequence
  REAGENT
  UNSURE 1..14
PPPATRRRRAVPIA

SEQ ID NO: 47 - protein, 14 aa, Artificial Sequence
  REAGENT
  UNSURE 1..14
PSPTNRSKRNLKME

SEQ ID NO: 48 - DNA, 12 bp, Artificial Sequence
  REAGENT
tcaaaagaaacc

SEQ ID NO: 49 - DNA, 12 bp, Artificial Sequence
  REAGENT
gctaaagctgct

SEQ ID NO: 50 - protein, 8 aa, Artificial Sequence
  REAGENT
  UNSURE 1..8
RKHXXRKH

SEQ ID NO: 51 - protein, 7 aa, Artificial Sequence
  REAGENT
  UNSURE 1..7
RKHXXKG

SEQ ID NO: 52 - protein, 9 aa, Artificial Sequence
  REAGENT
  UNSURE 1..9
CSVIQRSPR

SEQ ID NO: 53 - protein, 7 aa, Artificial Sequence
  REAGENT
  UNSURE 1..7
CAPRTPR

SEQ ID NO: 54 - protein, 5 aa, Artificial Sequence
  REAGENT
  UNSURE 1..5
PIPAR

SEQ ID NO: 55 - protein, 3 aa, Artificial Sequence
  REAGENT
  UNSURE 1..3
CPR

SEQ ID NO: 56 - protein, 6 aa, Artificial Sequence
  REAGENT
  UNSURE 1..6
CIKTAR

SEQ ID NO: 57 - protein, 5 aa, Artificial Sequence
  REAGENT
  UNSURE 1..5
CLQPR

SEQ ID NO: 58 - protein, 5 aa, Artificial Sequence
  REAGENT
  UNSURE 1..5
CSGIR

SEQ ID NO: 59 - protein, 6 aa, Artificial Sequence
  REAGENT
  UNSURE 1..6
CVRSPR

SEQ ID NO: 60 - protein, 6 aa, Artificial Sequence
  REAGENT
  UNSURE 1..6
CRTVVR

SEQ ID NO: 61 - protein, 9 aa, Artificial Sequence
  REAGENT
  UNSURE 1..9
CNHGNRQQC

SEQ ID NO: 62 - protein, 7 aa, Artificial Sequence
  REAGENT
  UNSURE 1..7
VVERVRR

SEQ ID NO: 63 - protein, 7 aa, Artificial Sequence
  REAGENT
  UNSURE 1..7
DKDKPLR

SEQ ID NO: 64 - protein, 7 aa, Artificial Sequence
  REAGENT
  UNSURE 1..7
GTWKQAR

SEQ ID NO: 65 - protein, 7 aa, Artificial Sequence
  REAGENT
  UNSURE 1..7
AVRRSAR

SEQ ID NO: 66 - protein, 7 aa, Artificial Sequence
  REAGENT
  UNSURE 1..7
AKGRSPR

SEQ ID NO: 67 - protein, 7 aa, Artificial Sequence
  REAGENT
  UNSURE 1..7
ARVRGYR

SEQ ID NO: 68 - protein, 7 aa, Artificial Sequence
  REAGENT
  UNSURE 1..7
RGVRGFR

SEQ ID NO: 69 - protein, 4 aa, Artificial Sequence
  REAGENT
  UNSURE 1..4
RTQR

SEQ ID NO: 70 - protein, 7 aa, Artificial Sequence
  REAGENT
  UNSURE 1..7
SIRRPPR

SEQ ID NO: 71 - protein, 7 aa, Artificial Sequence
  REAGENT
  UNSURE 1..7
RSRTQSR

SEQ ID NO: 72 - protein, 7 aa, Artificial Sequence
  REAGENT
  UNSURE 1..7
RPVRTSR

SEQ ID NO: 73 - protein, 1 aa, Artificial Sequence
  REAGENT
  UNSURE 1..1
R

SEQ ID NO: 74 - protein, 7 aa, Artificial Sequence
  REAGENT
  UNSURE 1..7
RLSRNPR

SEQ ID NO: 75 - protein, 7 aa, Artificial Sequence
  REAGENT
  UNSURE 1..7
RPTRMPR

SEQ ID NO: 76 - protein, 4 aa, Artificial Sequence
  REAGENT
  UNSURE 1..4
RGVR

SEQ ID NO: 77 - protein, 7 aa, Artificial Sequence
  REAGENT
  UNSURE 1..7
RIRRTDR

SEQ ID NO: 78 - protein, 7 aa, Artificial Sequence
  REAGENT
  UNSURE 1..7
RLQRVHR

SEQ ID NO: 79 - protein, 7 aa, Artificial Sequence
  REAGENT
  UNSURE 1..7
RPARPAR

SEQ ID NO: 80 - protein, 7 aa, Artificial Sequence
  REAGENT
  UNSURE 1..7
RGERPPR

SEQ ID NO: 81 - protein, 7 aa, Artificial Sequence
  REAGENT
  UNSURE 1..7
RVTRPPR

SEQ ID NO: 82 - protein, 5 aa, Artificial Sequence
  REAGENT
  UNSURE 1..5
CRPVR

SEQ ID NO: 83 - protein, 6 aa, Artificial Sequence
  REAGENT
  UNSURE 1..6
CSKTAR

SEQ ID NO: 84 - protein, 7 aa, Artificial Sequence
  REAGENT
  UNSURE 1..7
CSLRTPK

SEQ ID NO: 85 - protein, 5 aa, Artificial Sequence
  REAGENT
  UNSURE 1..5
CRKKR

SEQ ID NO: 86 - protein, 4 aa, Artificial Sequence
  REAGENT
  UNSURE 1..4
CRRR

SEQ ID NO: 87 - protein, 4 aa, Artificial Sequence
  REAGENT
  UNSURE 1..4
CRKR

SEQ ID NO: 88 - protein, 5 aa, Artificial Sequence
  REAGENT
  UNSURE 1..5
CRPRR

SEQ ID NO: 89 - protein, 6 aa, Artificial Sequence
  REAGENT
  UNSURE 1..6
CPKRDR

SEQ ID NO: 90 - protein, 7 aa, Artificial Sequence
  REAGENT
  UNSURE 1..7
CREKPER

SEQ ID NO: 91 - protein, 7 aa, Artificial Sequence
  REAGENT
  UNSURE 1..7
CMPKRER

SEQ ID NO: 92 - protein, 7 aa, Artificial Sequence
  REAGENT
  UNSURE 1..7
GGTRPVR

SEQ ID NO: 93 - protein, 7 aa, Artificial Sequence
  REAGENT
  UNSURE 1..7
RAVRSPR

SEQ ID NO: 94 - protein, 7 aa, Artificial Sequence
  REAGENT
  UNSURE 1..7
HTHRLPR

SEQ ID NO: 95 - protein, 7 aa, Artificial Sequence
  REAGENT
  UNSURE 1..7
VKGPARR

SEQ ID NO: 96 - protein, 7 aa, Artificial Sequence
  REAGENT
  UNSURE 1..7
IPVRSLR

SEQ ID NO: 97 - protein, 7 aa, Artificial Sequence
  REAGENT
  UNSURE 1..7
LRKYSTR

SEQ ID NO: 98 - protein, 5 aa, Artificial Sequence
  REAGENT
  UNSURE 1..5
DRGAR

SEQ ID NO: 99 - protein, 7 aa, Artificial Sequence
  REAGENT
  UNSURE 1..7
DRLRHAR

SEQ ID NO: 100 - protein, 7 aa, Artificial Sequence
  REAGENT
  UNSURE 1..7
GMGRKFR

SEQ ID NO: 101 - protein, 7 aa, Artificial Sequence
  REAGENT
  UNSURE 1..7
GRHSEVR

SEQ ID NO: 102 - protein, 7 aa, Artificial Sequence
  REAGENT
  UNSURE 1..7
RTVRAAR

SEQ ID NO: 103 - protein, 5 aa, Artificial Sequence
  REAGENT
  UNSURE 1..5
RGARR

SEQ ID NO: 104 - protein, 7 aa, Artificial Sequence
  REAGENT
  UNSURE 1..7
RSQRSAR

SEQ ID NO: 105 - protein, 7 aa, Artificial Sequence
  REAGENT
  UNSURE 1..7
REKRVTR

SEQ ID NO: 106 - protein, 7 aa, Artificial Sequence
  REAGENT
  UNSURE 1..7
RPGRSRR

SEQ ID NO: 107 - protein, 7 aa, Artificial Sequence
  REAGENT
  UNSURE 1..7
RRPRPAR

SEQ ID NO: 108 - protein, 7 aa, Artificial Sequence
  REAGENT
  UNSURE 1..7
RFVRQST

SEQ ID NO: 109 - protein, 7 aa, Artificial Sequence
  REAGENT
  UNSURE 1..7
RSGRAMR

SEQ ID NO: 110 - protein, 7 aa, Artificial Sequence
  REAGENT
  UNSURE 1..7
RGPRVSR

SEQ ID NO: 111 - protein, 7 aa, Artificial Sequence
  REAGENT
  UNSURE 1..7
RTVRNSR

SEQ ID NO: 112 - protein, 7 aa, Artificial Sequence
  REAGENT
  UNSURE 1..7
RPARPAK

SEQ ID NO: 113 - protein, 7 aa, Artificial Sequence
  REAGENT
  UNSURE 1..7
RPARPAA

SEQ ID NO: 114 - protein, 7 aa, Artificial Sequence
  REAGENT
  UNSURE 1..7
RPAKPAR

SEQ ID NO: 115 - protein, 7 aa, Artificial Sequence
  REAGENT
  UNSURE 1..7
APARPAR

SEQ ID NO: 116 - protein, 7 aa, Artificial Sequence
  REAGENT
  UNSURE 1..7
APAAPAR

SEQ ID NO: 117 - protein, 7 aa, Artificial Sequence
  REAGENT
  UNSURE 1..7
APARPAA

SEQ ID NO: 118 - protein, 7 aa, Artificial Sequence
  REAGENT
  UNSURE 1..7
RPAAPAA

SEQ ID NO: 119 - protein, 8 aa, Artificial Sequence
  REAGENT
  UNSURE 1..8
RPARPARK

SEQ ID NO: 120 - protein, 8 aa, Artificial Sequence
  REAGENT
  UNSURE 1..8
RPARPARN

SEQ ID NO: 121 - protein, 8 aa, Artificial Sequence
  REAGENT
  UNSURE 1..8
RPARPARI

SEQ ID NO: 122 - protein, 8 aa, Artificial Sequence
  REAGENT
  UNSURE 1..8
RPARPARP

SEQ ID NO: 123 - protein, 8 aa, Artificial Sequence
  REAGENT
  UNSURE 1..8
RPARPARS

SEQ ID NO: 124 - protein, 7 aa, Artificial Sequence
  REAGENT
  UNSURE 1..7
RGERPPR

SEQ ID NO: 125 - protein, 7 aa, Artificial Sequence
  REAGENT
  UNSURE 1..7
RVTRPPR

SEQ ID NO: 126 - protein, 8 aa, Artificial Sequence
  REAGENT
  UNSURE 1..8
CRCDKPRR

SEQ ID NO: 127 - protein, 9 aa, Artificial Sequence
  REAGENT
  UNSURE 1..9
CRCDKPRRA

SEQ ID NO: 128 - protein, 4 aa, Artificial Sequence
  REAGENT
  UNSURE 1..4
TKPR

SEQ ID NO: 129 - protein, 5 aa, Artificial Sequence
  REAGENT
  UNSURE 1..5
TKPPR

SEQ ID NO: 130 - protein, 7 aa, Artificial Sequence
  REAGENT
  UNSURE 1..7
ATWLPPR

SEQ ID NO: 131 - protein, 5 aa, Artificial Sequence
  REAGENT
  UNSURE 1..5
DDDDK

SEQ ID NO: 132 - protein, 7 aa, Artificial Sequence
  REAGENT
  UNSURE 1..7
RGARDIR

SEQ ID NO: 133 - protein, 5 aa, Artificial Sequence
  REAGENT
  UNSURE 1..5
RVSRR

SEQ ID NO: 134 - protein, 2 aa, Artificial Sequence
  REAGENT
  UNSURE 1..2
RM

SEQ ID NO: 135 - protein, 10 aa, Artificial Sequence
  REAGENT
  UNSURE 1..10
RVRRPARTSF

SEQ ID NO: 136 - protein, 12 aa, Artificial Sequence
  REAGENT
  UNSURE 1..12
RKFRRPPRRVLA

SEQ ID NO: 137 - protein, 11 aa, Artificial Sequence
  REAGENT
  UNSURE 1..11
RTMTRPARASV

SEQ ID NO: 138 - protein, 7 aa, Artificial Sequence
  REAGENT
  UNSURE 1..7
REVRPPR

SEQ ID NO: 139 - protein, 7 aa, Artificial Sequence
  REAGENT
  UNSURE 1..7
RHLRPAR

SEQ ID NO: 140 - protein, 10 aa, Artificial Sequence
  REAGENT
  UNSURE 1..10
RVKRPPRAER

SEQ ID NO: 141 - protein, 10 aa, Artificial Sequence
  REAGENT
  UNSURE 1..10
RPGRPPRFSA

SEQ ID NO: 142 - protein, 10 aa, Artificial Sequence
  REAGENT
  UNSURE 1..10
RAQRPARDHR

SEQ ID NO: 143 - protein, 1 aa, Artificial Sequence
  REAGENT
  UNSURE 1..1
R

SEQ ID NO: 144 - protein, 7 aa, Artificial Sequence
  REAGENT
  UNSURE 1..7
RAPRPAR

SEQ ID NO: 145 - protein, 10 aa, Artificial Sequence
  REAGENT
  UNSURE 1..10
RERRPARETT

SEQ ID NO: 146 - protein, 7 aa, Artificial Sequence
  REAGENT
  UNSURE 1..7
RGLRPAR

SEQ ID NO: 147 - protein, 10 aa, Artificial Sequence
  REAGENT
  UNSURE 1..10
RVYRPARNLR

SEQ ID NO: 148 - protein, 10 aa, Artificial Sequence
  REAGENT
  UNSURE 1..10
RVGRPARSRS

SEQ ID NO: 149 - protein, 7 aa, Artificial Sequence
  REAGENT
  UNSURE 1..7
RITRPAR

SEQ ID NO: 150 - protein, 7 aa, Artificial Sequence
  REAGENT
  UNSURE 1..7
RDRRPPR

SEQ ID NO: 151 - protein, 7 aa, Artificial Sequence
  REAGENT
  UNSURE 1..7
RFGRPPR

SEQ ID NO: 152 - protein, 10 aa, Artificial Sequence
  REAGENT
  UNSURE 1..10
RGTRPARWDR

SEQ ID NO: 153 - protein, 7 aa, Artificial Sequence
  REAGENT
  UNSURE 1..7
RGVRPPR

SEQ ID NO: 154 - protein, 10 aa, Artificial Sequence
  REAGENT
  UNSURE 1..10
RGVRPARSIH

SEQ ID NO: 155 - protein, 9 aa, Artificial Sequence
  REAGENT
  UNSURE 1..9
CGGGGGGGC

SEQ ID NO: 156 - protein, 9 aa, Artificial Sequence
  REAGENT
  UNSURE 1..9
CRGDKGPDC

SEQ ID NO: 157 - protein, 9 aa, Artificial Sequence
  REAGENT
  UNSURE 1..9
CRGDKGPDA

SEQ ID NO: 158 - protein, 9 aa, Artificial Sequence
  REAGENT
  UNSURE 1..9
CRGDKGPDG

SEQ ID NO: 159 - protein, 8 aa, Artificial Sequence
  REAGENT
  UNSURE 1..8
CRGDKGPD

SEQ ID NO: 160 - protein, 7 aa, Artificial Sequence
  REAGENT
  UNSURE 1..7
CRGDKGP

SEQ ID NO: 161 - protein, 4 aa, Artificial Sequence
  REAGENT
  UNSURE 1..4
CRGD

SEQ ID NO: 162 - protein, 3 aa, Artificial Sequence
  REAGENT
  UNSURE 1..3
CRG

SEQ ID NO: 163 - protein, 2 aa, Artificial Sequence
  REAGENT
  UNSURE 1..2
CR

SEQ ID NO: 164 - protein, 4 aa, Artificial Sequence
  REAGENT
  UNSURE 1..4
RPAR